European Patent Specification EP 3 802 557 B1, published August 6, 2025. Title: THERAPEUTIC TREATMENT OF MICROSATELLITE UNSTABLE CANCERS. Applicant: Broad Institute, Inc. Dana Farber Cancer Institute, Inc. The sequence listing filed with the application follows.

SEQUENCE LISTING (29 sequences)

SEQ ID NO: 1 - DNA, 20 bp, Artificial
  Synthetic
gtaaattggaaaacccacgg

SEQ ID NO: 2 - DNA, 20 bp, Artificial
  Synthetic
atcctgtggaacataccatg

SEQ ID NO: 3 - DNA, 20 bp, Artificial
  Synthetic
gtagcagtaagtgcaacgat

SEQ ID NO: 4 - DNA, 20 bp, Artificial
  Synthetic
agcacgtacataagcatcag

SEQ ID NO: 5 - DNA, 21 bp, Artificial
  Synthetic
cagcactgccaatggttccaa

SEQ ID NO: 6 - DNA, 21 bp, Artificial
  Synthetic
gccttaacagtctggttaaac

SEQ ID NO: 7 - DNA, 20 bp, Artificial
  Synthetic
tcgcctccaagaatgtaagt

SEQ ID NO: 8 - DNA, 21 bp, Artificial
  Synthetic
tctgcattttaactatggctc

SEQ ID NO: 9 - DNA, 21 bp, Artificial
  Synthetic
tgactacttttgacttcagcc

SEQ ID NO: 10 - DNA, 22 bp, Artificial
  Synthetic
aaccattcaacatttttaaccc

SEQ ID NO: 11 - DNA, 20 bp, Artificial
  Synthetic
aaacaggatgcctgccttta

SEQ ID NO: 12 - DNA, 20 bp, Artificial
  Synthetic
ggactttccacctatgggac

SEQ ID NO: 13 - DNA, 25 bp, Artificial
  Synthetic
agcagataagacagtattactagtt

SEQ ID NO: 14 - DNA, 23 bp, Artificial
  Synthetic
actcactctagtgataaatcggg

SEQ ID NO: 15 - DNA, 20 bp, Artificial
  Synthetic
ggaagaatcaaatagacaat

SEQ ID NO: 16 - DNA, 24 bp, Artificial
  Synthetic
gctggccatatatatatttaaacc

SEQ ID NO: 17 - DNA, 20 bp, Artificial
  Synthetic
ggtgtgcgtatgaagcagtg

SEQ ID NO: 18 - DNA, 20 bp, Artificial
  Synthetic
gcagtgctaaccttgcattg

SEQ ID NO: 19 - DNA, 20 bp, Artificial
  Synthetic
agagactgctgaggagtcca

SEQ ID NO: 20 - DNA, 20 bp, Artificial
  Synthetic
acaacgtcttggagcgccag

SEQ ID NO: 21 - DNA, 20 bp, Artificial
  Synthetic
tttggccagcataagccatg

SEQ ID NO: 22 - DNA, 20 bp, Artificial
  Synthetic
gccagcacatggtttaggag

SEQ ID NO: 23 - DNA, 21 bp, Artificial
  Synthetic
cgccagttagctcaatatcat

SEQ ID NO: 24 - DNA, 21 bp, Artificial
  Synthetic
ccgccagtatgttgtaagaaa

SEQ ID NO: 25 - DNA, 21 bp, Artificial
  Synthetic
ctcagttccagtacggctcca

SEQ ID NO: 26 - DNA, 21 bp, Artificial
  Synthetic
cagcactgggtatggttccaa

SEQ ID NO: 27 - DNA, 21 bp, Artificial
  Synthetic
gccttaactcactggttaaac

SEQ ID NO: 28 - DNA, 17 bp, Artificial
  Synthetic
attcgttggaaacggga

SEQ ID NO: 29 - DNA, 11 bp, Artificial
  Synthetic
gttagggttag